European Patent Specification EP 3 522 706 B1, published June 7, 2023. Title: BACILLUS THURINGIENSIS RTI545 COMPOSITIONS AND METHODS OF USE FOR BENEFITING PLANT GROWTH AND CONTROLLING PLANT PESTS. Applicant: FMC Corporation. The sequence listing filed with the application follows.

SEQUENCE LISTING (2 sequences)

SEQ ID NO: 1 - DNA, 1544 bp, Bacillus thuringiensis
agaaaggaggtgatccagccgcaccttccgatacggctaccttgttacgacttcaccccaatcatctgtcccaccttaggcggctggctccaaaaaggttaccccaccgacttcgggtgttacaaactctcgtggtgtgacgggcggtgtgtacaaggcccgggaacgtattcaccgcggcatgctgatccgcgattactagcgattccagcttcatgtaggcgagttgcagcctacaatccgaactgagaacggttttatgagattagctccacctcgcggtcttgcagctctttgtaccgtccattgtagcacgtgtgtagcccaggtcataaggggcatgatgatttgacgtcatccccaccttcctccggtttgtcaccggcagtcaccttagagtgcccaacttaatgatggcaactaagatcaagggttgcgctcgttgcgggacttaacccaacatctcacgacacgagctgacgacaaccatgcaccacctgtcactctgctcccgaaggagaagccctatctctagggttttcagaggatgtcaagacctggtaaggttcttcgcgttgcttcgaattaaaccacatgctccaccgcttgtgcgggcccccgtcaattcctttgagtttcagccttgcggccgtactccccaggcggagtgcttaatgcgttaacttcagcactaaagggcggaaaccctctaacacttagcactcatcgtttacggcgtggactaccagggtatctaatcctgtttgctccccacgctttcgcgcctcagtgtcagttacagaccagaaagtcgccttcgccactggtgttcctccatatctctacgcatttcaccgctacacatggaattccactttcctcttctgcactcaagtctcccagtttccaatgaccctccacggttgagccgtgggctttcacatcagacttaagaaaccacctgcgcgcgctttacgcccaataattccggataacgcttgccacctacgtattaccgcggctgctggcacgtagttagccgtggctttctggttaggtaccgtcaaggtgccagcttattcaactagcacttgttcttccctaacaacagagttttacgacccgaaagccttcatcactcacgcggcgttgctccgtcagactttcgtccattgcggaagattccctactgctgcctcccgtaggagtctgggccgtgtctcagtcccagtgtggccgatcaccctctcaggtcggctacgcatcgttgccttggtgagccgttacctcaccaactagctaatgcgacgcgggtccatccataagtgacagccgaagccgcctttcaatttcgaaccatgcagttcaaaatgttatccggtattagccccggtttcccggagttatcccagtcttatgggcaggttacccacgtgttactcacccgtccgccgctaacttcttgagagcaagctctcaatccattcgctcgacttgcatgtattaggcacgccgccagcgttcatcctgagccaggatcaaac

SEQ ID NO: 2 - DNA, 3534 bp, Bacillus thuringiensis
ttgacaggtcaactagttcaatacggacgccaccgccaacgaagaagttatgcccgtattagtgaagtattagagttaccaaatcttatcgaaattcaaacctcttcttatcagtggtttcttgatgagggtttgcgagaaatgttccaagacatttctccgattgaagactttacgggaaatctatcgcttgaatttatcgactacagcttaggtgaacctaaatactctgtagacgaatgcaaagagcgtgatgtgacgtatgcagcaccacttcgtgtaaaagtgcgtctaatcaacaaggaaactggtgaagtaaaagaacaagatgtgttcatgggagatttcccactcatgacagagactggaacattcgtaattaacggtgcagaacgtgttatcgtttcccagttagttcgctctccaagcgtatactatagtggcaaagtggataaaaacggaaaacgtggttttactgctactgtaattccaaaccgcggagcttggttagagtatgagacagatgctaaggatgttgtatatgtgcgtattgaccgtacgcgtaaacttcctgtaactgttttgttacgcgcattagggtttggctctgatcaagaaatcaccgagcttttaggtgataacgaatacttaagcaacacattagaaaaagacaacacagatagtacagaaaaagcattgcttgaaatttatgagcgtctacgtcctggtgaaccaccaacagtagaaaatgctaagagcttacttgtgtctcgtttcttcgatccaaagcgctacgatttagcaaatgtaggtcgctataagatcaacaagaagttacacattaaaaacagattgtttaatcaacgtttagctgaaacattagtggatccagaaactggtgaaattttagcggcagaaggaacaatcttagatcgtcgtacacttgatcgcattttaccttacttagagaaaaacattggattcaaaacagcgaaaccaatgggtggagtggtagaaggcgatgttgagctgcaatctattaagatttatgctcctgagtcggaaggcgaacgtgtaattaatgtaattggtaatgcaaatattactcgtgatgtgaaacacatcacaccaggtgatatccttgcttctatcagttacttcttcaacctactatacaaagtaggggatacagatgatattgaccatttaggaaaccgtcgtctgcgttctgttggagaactattacaaaatcaattccgtatcggtctttctcgtatggaacgtgttgttcgtgagagaatgtcgatccaagatacaaatgcaattacaccacaggcgctaattaatattcgtcctgttattgcatctattaaagagttcttcggaagttctcagttatctcagttcatggaccaaacaaatccattagcagagttaactcacaaacgaagactatctgcattaggacctggtggtttaacgcgtgagcgcgcaggctttgaagtacgtgacgttcattactcccactacggtcgtatgtgtccgattgaaacaccagagggaccaaacatcggtttgattaactcattatcttcgttcgcgaaagtaaatgagtttggtttcattgaaacaccatatcgtcgtgttgacccagaaactggtcttgtaacagggcatgttgattatttaacagcagatgaagaagataactatgttgtagcccaagcgaatatgaaattatctgatgaaggtgaattcctaagtgaagatatcgtagctcgtttccgtggtgaaaacattgtcacaaatagagaacgcatcgactacatggatgtatctccaaaacaagtagtgtcggcagcgacagcttgtattccgttcttagaaaacgatgactctaaccgcgcacttatgggagcgaacatgcaacgtcaggcggttccgttaatgaatccggaatctccgattgtaggtacaggtatggagtacgtatcagcaaaagactcaggtgctgcagtaatctgtaaacatcctggtgttgttgagcgcgtagaagcacgtgaagtttgggtacgtcgctatgtagaagttgacggtcaaacagtaaaaggcgacttagatcgctacaaaatgcaaaaattcattcgttctaaccaaggaacttgttacaaccaacgtccaatcgtaagtgttggaaatgaagttgtaaaaggtgaaatccttgcggatggtccttctatggaattaggtgaactagcacttggacgtaacgtgcttgttggcttcatgacttgggacggttataactacgaggatgcgatcatcatgagtgagcgccttgtaaaagatgatgtgtacacttctattcatattgaagaatatgaatcagaagctcgtgatacgaagcttggaccagaagaaattacacgtgacattccaaatgttggggaagacgcattacgtaaccttgacgagcgcggtatcattcgcgttggtgctgaagtaaaagatggagatttacttgttggtaaagtaacacctaaaggtgtaacagaattaacagctgaagaacgtctattacatgctatctttggagaaaaagcgcgtgaagtacgtgatacatcactacgtgtaccacacggtggtggcggtattatcttagacgtaaaagtattcaaccgtgaagatggcgatgaattgccaccaggcgtgaatcaacttgtacgtgcatatatcgttcaaaaacgtaaaatttctgaaggtgacaagatggccggacgtcacggtaacaaaggtgttatttctcgtattttaccagaagaagatatgccttacttaccagacggtacgccaatcgatatcatgttaaacccattaggggtaccatctcgtatgaatatcggtcaggtattagagcttcatcttggtatggcagcaagatacctgggcattcacattgcaacaccagtattcgatggtgctcgtgaggaagatgtttggggcacaattgaagaagctggtatggcaaatgacgcgaaaacaatcctgtatgacggacgtactggtgaaccattcgataaccgcgtatctgttggtgtcatgtatatgatcaaacttgcgcacatggttgacgataaacttcatgctcgttctactggaccatactcacttgtaacgcagcaacctcttggaggtaaagctcagttcggtggacagcgtttcggtgagatggaggtttgggcacttgaagcttacggtgctgcttatactcttcaagaaatcttaacagtgaagtctgatgatgttgttggacgtgttaagacttatgaagcaattgttaaaggcgaaaatgttccagaaccaggcgttcctgaatcattcaaagtattgattaaagagctgcaaagtttaggtatggacgttaaaatgatgtctagcgacgatacagaaattgaaatgcgtgatacagaagatgacgatgatcatcaatcagcagataaattgaatgtcgaagttgagacaactaaggaataa